European Patent Application EP 4 328 238 A1, published February 28, 2024. Title: Proteins for use in the treatment of complement dysregulation disorders. Applicant: Ustav organicke chemie a biochemie AV CR, v. v. i. Application EP. The sequence listing filed with the application follows.

SEQUENCE LISTING (10 sequences)

SEQ ID NO: 1 - protein, 387 aa, synthetic construct
MMKYLLVFAIIATRIPVLLVIGSEDNRVPGDKKLTKEGAAALCKMKHLADKVAKERSQELKDRTQNFAGYIEFELYRIDYWLEKLNGPKGRKDGYAKLSDSDIEKVKEIFNKAKDGITKQLPEAKKAGEEAGKLHTEVKKAAENARGQDLDDDTAKSTGLYRVLNWYCITKEERHNATPNCDGIQFRKHYLSVNRSAIDCSSTSYEENYDWSANALQVALNSWEDVKPKKLESAGSDKNCNIGQSSESHPCTMTEEWQTPYKETVEKLRELEDAYQRGKKAHDAMLGYANTAYAVNTKVEQEKPLTEVIAAAKEAGKKGAKIIIPAAAPATPTNSTKNDDSAPTEHVDRGIATNETQVEVGIDADFDSLLDATEAAEVTRRHQRTAM

SEQ ID NO: 2 - protein, 28 aa, synthetic construct
YIEFELYRIDYWLEKLNGPKGRKDGYAK

SEQ ID NO: 3 - protein, 4 aa, synthetic construct
DWSA

SEQ ID NO: 4 - protein, 13 aa, synthetic construct
NTAYAVNTKVEQE

SEQ ID NO: 5 - protein, 346 aa, synthetic construct
LLVIGSEDNRVPGDKKLTKEGAAALCKMKHLADKVAKERSQELKDRTQNFAGYIEFELYRIDYWLEKLNGPKGRKDGYAKLSDSDIEKVKEIFNKAKDGITKQLPEAKKAGEEAGKLHTEVKKAAENARGQDLDDDTAKSTGLYRVLNWYCITKEERHNATPNCDGIQFRKHYLSVNRSAIDCSSTSYEENYDWSANALQVALNSWEDVKPKKLESAGSDKNCNIGQSSESHPCTMTEEWQTPYKETVEKLRELEDAYQRGKKAHDAMLGYANTAYAVNTKVEQEKPLTEVIAAAKEAGKKGAKIIIPAAAPATPTNSTKNDDSAPTEHVDRGIATNETQVEVGID

SEQ ID NO: 6 - protein, 365 aa, synthetic construct
MMKYLLVFAIIATRIPVLLVIGSEDNRVPGDKKLTKEGAAALCKMKHLADKVAKERSQELKDRTQNFAGYIEFELYRIDYWLEKLNGPKGRKDGYAKLSDSDIEKVKEIFNKAKDGITKQLPEAKKAGEEAGKLHTEVKKAAENARGQDLDDDTAKSTGLYRVLNWYCITKEERHNATPNCDGIQFRKHYLSVNRSAIDCSSTSYEENYDWSANALQVALNSWEDVKPKKLESAGSDKNCNIGQSSESHPCTMTEEWQTPYKETVEKLRELEDAYQRGKKAHDAMLGYANTAYAVNTKVEQEKPLTEVIAAAKEAGKKGAKIIIPAAAPATPTNSTKNDDSAPTEHVDRGIATNETQVEVGIDAD

SEQ ID NO: 7 - protein, 286 aa, synthetic construct
SEDNRVPGDKKLTKEGAAALCKMKHLADKVAKERSQELKDRTQNFAGYIEFELYRIDYWLEKLNGPKGRKDGYAKLSDSDIEKVKEIFNKAKDGITKQLPEAKKAGEEAGKLHTEVKKAAENARGQDLDDDTAKSTGLYRVLNWYCITKEERHNATPNCDGIQFRKHYLSVNRSAIDCSSTSYEENYDWSANALQVALNSWEDVKPKKLESAGSDKNCNIGQSSESHPCTMTEEWQTPYKETVEKLRELEDAYQRGKKAHDAMLGYANTAYAVNTKVEQEKPLTEV

SEQ ID NO: 8 - protein, 234 aa, synthetic construct
GYIEFELYRIDYWLEKLNGPKGRKDGYAKLSDSDIEKVKEIFNKAKDGITKQLPEAKKAGEEAGKLHTEVKKAAENARGQDLDDDTAKSTGLYRVLNWYCITKEERHNATPNCDGIQFRKHYLSVNRSAIDCSSTSYEENYDWSANALQVALNSWEDVKPKKLESAGSDKNCNIGQSSESHPCTMTEEWQTPYKETVEKLRELEDAYQRGKKAHDAMLGYANTAYAVNTKVEQE

SEQ ID NO: 9 - DNA, 1104 bp, synthetic construct
  source 1..1104: mol_type = other DNA
atgggcagcagccatcatcatcatcatcacagcagcggcctggtgccgcgcggcagccatatgttgttagtaattggcagtgaggataaccgtgttccaggagacaagaagttgacgaaagagggagcagcggcactctgtaaaatgaagcatcttgctgataaagttgcaaaggagagatcacaagagttaaaggatagaactcaaaattttgctggttatatagagttcgagttgtatagaatagattattggttggaaaagctgaacggtccgaaggggcgaaaagacggttatgctaagctgtctgactctgatatagaaaaagtaaaggagatattcaacaaggcaaaagatggaataactaagcaactccctgaggcaaagaaagccggtgaggaagctggaaaactacatactgaagtgaagaaggccgcggagaatgcacgtggacaggatcttgatgacgatacggcgaagtccactggcttgtacagggtgctgaattggtactgcattactaaagaagaaaggcacaacgctacccctaactgtgacggaatccaattcagaaagcattatctgtcggtgaatagaagcgctattgactgcagcagcaccagctatgaggagaattatgattggtctgcgaacgcgctgcaggtggccttaaatagctgggaggatgtgaagccaaaaaaattggagtcagccgggtcggacaagaattgcaacatcggccaatcttccgagagccatccatgcaccatgacagaggagtggcagactccatacaaggaaactgtcgaaaagctaagggaacttgaggatgcgtaccaaaggggcaagaaggctcatgatgctatgttgggttacgctaataccgcatatgctgtgaacacgaaagtggaacaggaaaagccgctgacagaggtgatagcggcagctaaggaagcagggaaaaagggcgcgaaaattataatacccgcagctgccccagcaacaccgactaacagcacaaaaaatgatgatagtgctccaaccgagcatgttgatagagggattgcaacaaatgaaacacaggtggaagttggtattgattaa

SEQ ID NO: 10 - protein, 367 aa, synthetic construct
MGSSHHHHHHSSGLVPRGSHMLLVIGSEDNRVPGDKKLTKEGAAALCKMKHLADKVAKERSQELKDRTQNFAGYIEFELYRIDYWLEKLNGPKGRKDGYAKLSDSDIEKVKEIFNKAKDGITKQLPEAKKAGEEAGKLHTEVKKAAENARGQDLDDDTAKSTGLYRVLNWYCITKEERHNATPNCDGIQFRKHYLSVNRSAIDCSSTSYEENYDWSANALQVALNSWEDVKPKKLESAGSDKNCNIGQSSESHPCTMTEEWQTPYKETVEKLRELEDAYQRGKKAHDAMLGYANTAYAVNTKVEQEKPLTEVIAAAKEAGKKGAKIIIPAAAPATPTNSTKNDDSAPTEHVDRGIATNETQVEVGID